European Patent Application EP 4 509 598 A1, published February 19, 2025. Title: FUCOSIDASE MUTANTS AND THE USE THEREOF. Applicant: CHO PHARMA, INC. Application US. The sequence listing filed with the application follows.

SEQUENCE LISTING (38 sequences)

SEQ ID NO: 1 - protein, 344 aa, Lactobacillus casei
MNDNVAWFKQAKYGMMIHWGLYSLLAGEYRGESSSAYAEWIQSKFQIPNAEYGNLATAFNPLYFDAKKIVALAKQCGMQYLVVTTKHHDGFAMYHSKVDAYNVYDATPFHRDIIGELAEACQKAGLKFGLYYSQDLDWHDPNGGGYKSNDVETAGTTWDNSWDFPDEDQKNFDLCFDNKILPQIKEIMSNYGDIATAWFDVPMTLSEAQSQTIYDTVRELQPNCLINSRLGNGKYDFVSLGDNEIPKNKEDMNKTDVDYNEITGFKPSPLGLYETAGTINDSWGFSYHDQNWKTPRTLYRYKQHLNDFGINYLLNVGLDPLGRVPMMAEENLLAAKALEDEANR

SEQ ID NO: 2 - protein, 344 aa, Artificial Sequence
MNDNVAWFKQAKYGMMIHWGLYSLLAGEYRGESSSAYAEWIQSKFQIPNAEYGNLATAFNPLYFDAKKIVALAKQCGMQYLVVTTKHHDGFAMYHSKVDAYNVYDATPFHRDIIGELAEACQKAGLKFGLYYSQDLDWHDPNGGGYKSNDVETAGTTWDNSWDFPDEDQKNFDLCFDNKILPQIKEIMSNYGDIATAWFDVPMTLSEAQSQTIYDTVRELQPNCLINSRLGNGKYDFVSLGDNEIPDNKEDMNKTDVDYNEITGFKPSPLGLYETAGTINDSWGFSYHDQNWKTPRTLYRYKQHLNDFGINYLLNVGLDPLGRVPMMAEENLLAAKALEDEANR

SEQ ID NO: 3 - protein, 344 aa, Artificial Sequence
MNDNVAWFKQAKYGMMIHWGLYSLLAGEYRGESSSAYAEWIQSKFQIPNAEYGNLATAFNPLYFDAKKIVALAKQCGMQYLVVTTKHHDGFAMYHSKVDAYNVYDATPFHRDIIGELAEACQKAGLKFGLYYSQDLDWHDPNGGGYKSNDVETAGTTWDNSWDFPDEDQKNFDLCFDNKILPQIKEIMSNYGDIATAWFDVPMTLSEAQSQTIYDTVRELQPNCLINSRLGNGKYDFVSLGDNEIPENKEDMNKTDVDYNEITGFKPSPLGLYETAGTINDSWGFSYHDQNWKTPRTLYRYKQHLNDFGINYLLNVGLDPLGRVPMMAEENLLAAKALEDEANR

SEQ ID NO: 4 - protein, 344 aa, Artificial Sequence
MNDNVAWFKQAKYGMMIHWGLYSLLAGEYRGESSSAYAEWIQSKFQIPNAEYGNLATAFNPLYFDAKKIVALAKQCGMQYLVVTTKHHDGFAMYHSKVDAYNVYDATPFHRDIIGELAEACQKAGLKFGLYYSQDLDWHDPNGGGYKSNDVETAGTTWDNSWDFPDEDQKNFDLCFDNKILPQIKEIMSNYGDIATAWFDVPMTLSEAQSQTIYDTVRELQPNCLINSRLGNGKYDFVSLGDNEIPFNKEDMNKTDVDYNEITGFKPSPLGLYETAGTINDSWGFSYHDQNWKTPRTLYRYKQHLNDFGINYLLNVGLDPLGRVPMMAEENLLAAKALEDEANR

SEQ ID NO: 5 - protein, 344 aa, Artificial Sequence
MNDNVAWFKQAKYGMMIHWGLYSLLAGEYRGESSSAYAEWIQSKFQIPNAEYGNLATAFNPLYFDAKKIVALAKQCGMQYLVVTTKHHDGFAMYHSKVDAYNVYDATPFHRDIIGELAEACQKAGLKFGLYYSQDLDWHDPNGGGYKSNDVETAGTTWDNSWDFPDEDQKNFDLCFDNKILPQIKEIMSNYGDIATAWFDVPMTLSEAQSQTIYDTVRELQPNCLINSRLGNGKYDFVSLGDNEIPANKEDMNKTDVDYNEITGFKPSPLGLYETAGTINDSWGFSYHDQNWKTPRTLYRYKQHLNDFGINYLLNVGLDPLGRVPMMAEENLLAAKALEDEANR

SEQ ID NO: 6 - protein, 344 aa, Artificial Sequence
MNDNVAWFKQAKYGMMIHWGLYSLLAGEYRGESSSAYAEWIQSKFQIPNAEYGNLATAFNPLYFDAKKIVALAKQCGMQYLVVTTKHHDGFAMYHSKVDAYNVYDATPFHRDIIGELAEACQKAGLKFGLYYSQDLDWHDPNGGGYKSNDVETAGTTWDNSWDFPDEDQKNFDLCFDNKILPQIKEIMSNYGDIATAWFDVPMTLSEAQSQTIYDTVRELQPNCLINSRLGNGKYDFVSLGDNEIPCNKEDMNKTDVDYNEITGFKPSPLGLYETAGTINDSWGFSYHDQNWKTPRTLYRYKQHLNDFGINYLLNVGLDPLGRVPMMAEENLLAAKALEDEANR

SEQ ID NO: 7 - protein, 344 aa, Artificial Sequence
MNDNVAWFKQAKYGMMIHWGLYSLLAGEYRGESSSAYAEWIQSKFQIPNAEYGNLATAFNPLYFDAKKIVALAKQCGMQYLVVTTKHHDGFAMYHSKVDAYNVYDATPFHRDIIGELAEACQKAGLKFGLYYSQDLDWHDPNGGGYKSNDVETAGTTWDNSWDFPDEDQKNFDLCFDNKILPQIKEIMSNYGDIATAWFDVPMTLSEAQSQTIYDTVRELQPNCLINSRLGNGKYDFVSLGDNEIPGNKEDMNKTDVDYNEITGFKPSPLGLYETAGTINDSWGFSYHDQNWKTPRTLYRYKQHLNDFGINYLLNVGLDPLGRVPMMAEENLLAAKALEDEANR

SEQ ID NO: 8 - protein, 344 aa, Artificial Sequence
MNDNVAWFKQAKYGMMIHWGLYSLLAGEYRGESSSAYAEWIQSKFQIPNAEYGNLATAFNPLYFDAKKIVALAKQCGMQYLVVTTKHHDGFAMYHSKVDAYNVYDATPFHRDIIGELAEACQKAGLKFGLYYSQDLDWHDPNGGGYKSNDVETAGTTWDNSWDFPDEDQKNFDLCFDNKILPQIKEIMSNYGDIATAWFDVPMTLSEAQSQTIYDTVRELQPNCLINSRLGNGKYDFVSLGDNEIPINKEDMNKTDVDYNEITGFKPSPLGLYETAGTINDSWGFSYHDQNWKTPRTLYRYKQHLNDFGINYLLNVGLDPLGRVPMMAEENLLAAKALEDEANR

SEQ ID NO: 9 - protein, 344 aa, Artificial Sequence
MNDNVAWFKQAKYGMMIHWGLYSLLAGEYRGESSSAYAEWIQSKFQIPNAEYGNLATAFNPLYFDAKKIVALAKQCGMQYLVVTTKHHDGFAMYHSKVDAYNVYDATPFHRDIIGELAEACQKAGLKFGLYYSQDLDWHDPNGGGYKSNDVETAGTTWDNSWDFPDEDQKNFDLCFDNKILPQIKEIMSNYGDIATAWFDVPMTLSEAQSQTIYDTVRELQPNCLINSRLGNGKYDFVSLGDNEIPLNKEDMNKTDVDYNEITGFKPSPLGLYETAGTINDSWGFSYHDQNWKTPRTLYRYKQHLNDFGINYLLNVGLDPLGRVPMMAEENLLAAKALEDEANR

SEQ ID NO: 10 - protein, 344 aa, Artificial Sequence
MNDNVAWFKQAKYGMMIHWGLYSLLAGEYRGESSSAYAEWIQSKFQIPNAEYGNLATAFNPLYFDAKKIVALAKQCGMQYLVVTTKHHDGFAMYHSKVDAYNVYDATPFHRDIIGELAEACQKAGLKFGLYYSQDLDWHDPNGGGYKSNDVETAGTTWDNSWDFPDEDQKNFDLCFDNKILPQIKEIMSNYGDIATAWFDVPMTLSEAQSQTIYDTVRELQPNCLINSRLGNGKYDFVSLGDNEIPMNKEDMNKTDVDYNEITGFKPSPLGLYETAGTINDSWGFSYHDQNWKTPRTLYRYKQHLNDFGINYLLNVGLDPLGRVPMMAEENLLAAKALEDEANR

SEQ ID NO: 11 - protein, 344 aa, Artificial Sequence
MNDNVAWFKQAKYGMMIHWGLYSLLAGEYRGESSSAYAEWIQSKFQIPNAEYGNLATAFNPLYFDAKKIVALAKQCGMQYLVVTTKHHDGFAMYHSKVDAYNVYDATPFHRDIIGELAEACQKAGLKFGLYYSQDLDWHDPNGGGYKSNDVETAGTTWDNSWDFPDEDQKNFDLCFDNKILPQIKEIMSNYGDIATAWFDVPMTLSEAQSQTIYDTVRELQPNCLINSRLGNGKYDFVSLGDNEIPNNKEDMNKTDVDYNEITGFKPSPLGLYETAGTINDSWGFSYHDQNWKTPRTLYRYKQHLNDFGINYLLNVGLDPLGRVPMMAEENLLAAKALEDEANR

SEQ ID NO: 12 - protein, 344 aa, Artificial Sequence
MNDNVAWFKQAKYGMMIHWGLYSLLAGEYRGESSSAYAEWIQSKFQIPNAEYGNLATAFNPLYFDAKKIVALAKQCGMQYLVVTTKHHDGFAMYHSKVDAYNVYDATPFHRDIIGELAEACQKAGLKFGLYYSQDLDWHDPNGGGYKSNDVETAGTTWDNSWDFPDEDQKNFDLCFDNKILPQIKEIMSNYGDIATAWFDVPMTLSEAQSQTIYDTVRELQPNCLINSRLGNGKYDFVSLGDNEIPPNKEDMNKTDVDYNEITGFKPSPLGLYETAGTINDSWGFSYHDQNWKTPRTLYRYKQHLNDFGINYLLNVGLDPLGRVPMMAEENLLAAKALEDEANR

SEQ ID NO: 13 - protein, 344 aa, Artificial Sequence
MNDNVAWFKQAKYGMMIHWGLYSLLAGEYRGESSSAYAEWIQSKFQIPNAEYGNLATAFNPLYFDAKKIVALAKQCGMQYLVVTTKHHDGFAMYHSKVDAYNVYDATPFHRDIIGELAEACQKAGLKFGLYYSQDLDWHDPNGGGYKSNDVETAGTTWDNSWDFPDEDQKNFDLCFDNKILPQIKEIMSNYGDIATAWFDVPMTLSEAQSQTIYDTVRELQPNCLINSRLGNGKYDFVSLGDNEIPQNKEDMNKTDVDYNEITGFKPSPLGLYETAGTINDSWGFSYHDQNWKTPRTLYRYKQHLNDFGINYLLNVGLDPLGRVPMMAEENLLAAKALEDEANR

SEQ ID NO: 14 - protein, 344 aa, Artificial Sequence
MNDNVAWFKQAKYGMMIHWGLYSLLAGEYRGESSSAYAEWIQSKFQIPNAEYGNLATAFNPLYFDAKKIVALAKQCGMQYLVVTTKHHDGFAMYHSKVDAYNVYDATPFHRDIIGELAEACQKAGLKFGLYYSQDLDWHDPNGGGYKSNDVETAGTTWDNSWDFPDEDQKNFDLCFDNKILPQIKEIMSNYGDIATAWFDVPMTLSEAQSQTIYDTVRELQPNCLINSRLGNGKYDFVSLGDNEIPSNKEDMNKTDVDYNEITGFKPSPLGLYETAGTINDSWGFSYHDQNWKTPRTLYRYKQHLNDFGINYLLNVGLDPLGRVPMMAEENLLAAKALEDEANR

SEQ ID NO: 15 - protein, 344 aa, Artificial Sequence
MNDNVAWFKQAKYGMMIHWGLYSLLAGEYRGESSSAYAEWIQSKFQIPNAEYGNLATAFNPLYFDAKKIVALAKQCGMQYLVVTTKHHDGFAMYHSKVDAYNVYDATPFHRDIIGELAEACQKAGLKFGLYYSQDLDWHDPNGGGYKSNDVETAGTTWDNSWDFPDEDQKNFDLCFDNKILPQIKEIMSNYGDIATAWFDVPMTLSEAQSQTIYDTVRELQPNCLINSRLGNGKYDFVSLGDNEIPTNKEDMNKTDVDYNEITGFKPSPLGLYETAGTINDSWGFSYHDQNWKTPRTLYRYKQHLNDFGINYLLNVGLDPLGRVPMMAEENLLAAKALEDEANR

SEQ ID NO: 16 - protein, 344 aa, Artificial Sequence
MNDNVAWFKQAKYGMMIHWGLYSLLAGEYRGESSSAYAEWIQSKFQIPNAEYGNLATAFNPLYFDAKKIVALAKQCGMQYLVVTTKHHDGFAMYHSKVDAYNVYDATPFHRDIIGELAEACQKAGLKFGLYYSQDLDWHDPNGGGYKSNDVETAGTTWDNSWDFPDEDQKNFDLCFDNKILPQIKEIMSNYGDIATAWFDVPMTLSEAQSQTIYDTVRELQPNCLINSRLGNGKYDFVSLGDNEIPVNKEDMNKTDVDYNEITGFKPSPLGLYETAGTINDSWGFSYHDQNWKTPRTLYRYKQHLNDFGINYLLNVGLDPLGRVPMMAEENLLAAKALEDEANR

SEQ ID NO: 17 - protein, 344 aa, Artificial Sequence
MNDNVAWFKQAKYGMMIHWGLYSLLAGEYRGESSSAYAEWIQSKFQIPNAEYGNLATAFNPLYFDAKKIVALAKQCGMQYLVVTTKHHDGFAMYHSKVDAYNVYDATPFHRDIIGELAEACQKAGLKFGLYYSQDLDWHDPNGGGYKSNDVETAGTTWDNSWDFPDEDQKNFDLCFDNKILPQIKEIMSNYGDIATAWFDVPMTLSEAQSQTIYDTVRELQPNCLINSRLGNGKYDFVSLGDNEIPWNKEDMNKTDVDYNEITGFKPSPLGLYETAGTINDSWGFSYHDQNWKTPRTLYRYKQHLNDFGINYLLNVGLDPLGRVPMMAEENLLAAKALEDEANR

SEQ ID NO: 18 - protein, 344 aa, Artificial Sequence
MNDNVAWFKQAKYGMMIHWGLYSLLAGEYRGESSSAYAEWIQSKFQIPNAEYGNLATAFNPLYFDAKKIVALAKQCGMQYLVVTTKHHDGFAMYHSKVDAYNVYDATPFHRDIIGELAEACQKAGLKFGLYYSQDLDWHDPNGGGYKSNDVETAGTTWDNSWDFPDEDQKNFDLCFDNKILPQIKEIMSNYGDIATAWFDVPMTLSEAQSQTIYDTVRELQPNCLINSRLGNGKYDFVSLGDNEIPYNKEDMNKTDVDYNEITGFKPSPLGLYETAGTINDSWGFSYHDQNWKTPRTLYRYKQHLNDFGINYLLNVGLDPLGRVPMMAEENLLAAKALEDEANR

SEQ ID NO: 19 - DNA, 27 bp, Artificial Sequence
  source 1..27: mol_type = other DNA
gcgaacaaagaagatatgaacaagacc

SEQ ID NO: 20 - DNA, 27 bp, Artificial Sequence
  source 1..27: mol_type = other DNA
tgcaacaaagaagatatgaacaagacc

SEQ ID NO: 21 - DNA, 27 bp, Artificial Sequence
  source 1..27: mol_type = other DNA
gataacaaagaagatatgaacaagacc

SEQ ID NO: 22 - DNA, 27 bp, Artificial Sequence
  source 1..27: mol_type = other DNA
gaaaacaaagaagatatgaacaagacc

SEQ ID NO: 23 - DNA, 27 bp, Artificial Sequence
  source 1..27: mol_type = other DNA
tttaacaaagaagatatgaacaagacc

SEQ ID NO: 24 - DNA, 27 bp, Artificial Sequence
  source 1..27: mol_type = other DNA
ggcaacaaagaagatatgaacaagacc

SEQ ID NO: 25 - DNA, 27 bp, Artificial Sequence
  source 1..27: mol_type = other DNA
cataacaaagaagatatgaacaagacc

SEQ ID NO: 26 - DNA, 27 bp, Artificial Sequence
  source 1..27: mol_type = other DNA
attaacaaagaagatatgaacaagacc

SEQ ID NO: 27 - DNA, 27 bp, Artificial Sequence
  source 1..27: mol_type = other DNA
ctgaacaaagaagatatgaacaagacc

SEQ ID NO: 28 - DNA, 27 bp, Artificial Sequence
  source 1..27: mol_type = other DNA
atgaacaaagaagatatgaacaagacc

SEQ ID NO: 29 - DNA, 27 bp, Artificial Sequence
  source 1..27: mol_type = other DNA
aacaacaaagaagatatgaacaagacc

SEQ ID NO: 30 - DNA, 27 bp, Artificial Sequence
  source 1..27: mol_type = other DNA
ccgaacaaagaagatatgaacaagacc

SEQ ID NO: 31 - DNA, 27 bp, Artificial Sequence
  source 1..27: mol_type = other DNA
cagaacaaagaagatatgaacaagacc

SEQ ID NO: 32 - DNA, 27 bp, Artificial Sequence
  source 1..27: mol_type = other DNA
cgtaacaaagaagatatgaacaagacc

SEQ ID NO: 33 - DNA, 27 bp, Artificial Sequence
  source 1..27: mol_type = other DNA
agcaacaaagaagatatgaacaagacc

SEQ ID NO: 34 - DNA, 27 bp, Artificial Sequence
  source 1..27: mol_type = other DNA
accaacaaagaagatatgaacaagacc

SEQ ID NO: 35 - DNA, 27 bp, Artificial Sequence
  source 1..27: mol_type = other DNA
gtgaacaaagaagatatgaacaagacc

SEQ ID NO: 36 - DNA, 27 bp, Artificial Sequence
  source 1..27: mol_type = other DNA
tggaacaaagaagatatgaacaagacc

SEQ ID NO: 37 - DNA, 27 bp, Artificial Sequence
  source 1..27: mol_type = other DNA
tataacaaagaagatatgaacaagacc

SEQ ID NO: 38 - DNA, 21 bp, Artificial Sequence
  source 1..21: mol_type = other DNA
cgggatctcgttatcgcccag